European Patent Application EP 4 566 633 A1, published June 11, 2025. Title: An antibody-drug conjugate comprising a Toll like receptor 7/8 dual agonist compound. Applicant: アステラス製薬株式会社. The sequence listing filed with the application follows.

SEQUENCE LISTING (8 sequences)

SEQ ID NO: 1 - DNA, 1341 bp, synthetic construct
  source 1..1341: mol_type = other DNA
caggtgcagctggtggaatctggtggcggagttgttcagcctggcggctctctgagactgtcctgcaaggcttccggctactccttcaccggctacaccatgaactgggtccgacaggctcctggcaaaggcctggaatgggtcggactgatcaacccctataacggcggcaccatctacaaccagaagttcaagggcagattcaccctgtccgtggacaagtccaagtccaccgcctacctgcagatgaactccctgagagccgaggacaccgccgtgtactactgcgctagagactacggcttcgtgctggactattggggcagaggcacactggtcaccgtgtcctctgctagcacaaagggacctagcgtatttccattggctcctagcagcaaatccacaagtggtggaactgctgcactgggttgtctggttaaggattatttcccagagccagtcacagtttcctggaactctggggcactgacctccggagtgcacacattcccagccgtacttcaatccagtggtctctacagcctttcttcagtagtaaccgttccatcttctagcctcggaacccaaacttatatttgcaatgtgaatcacaagccttctaacactaaggttgataaacgagtcgaaccaaaatcctgcgataagacccacacttgcccaccttgccccgcaccagaattgttgggtggaccctctgtgttcctctttccacctaaacctaaggacactcttatgatctcacgcactcctgaagtaacctgtgtagtagtagacgtaagccatgaagaccccgaagtgaagttcaactggtatgttgatggtgtcgaagtgcataatgccaagactaaaccccgagaagaacagtataattctacttatagagtggtgtcagtgttgacagttctgcaccaagattggctcaatggtaaggagtacaaatgcaaggtgtcaaacaaggcactgccagcccctattgaaaagaccatcagcaaggccaagggccaacctcgagagccacaagtctacactctccctccttcacgtgaggagatgactaagaatcaggtttctctgacatgtttggtaaagggtttctacccaagcgacatagctgtggagtgggaatctaatggtcaaccagagaacaattacaaaaccaccccacccgttctcgactctgacggcagtttcttcctgtatagcaaacttactgtggataaatcccgatggcaacaaggcaacgtcttttcttgttccgtgatgcatgaggcacttcataaccactatacacaaaagagtttgtctttgtctccaggaaaa

SEQ ID NO: 2 - protein, 447 aa, synthetic construct
QVQLVESGGGVVQPGGSLRLSCKASGYSFTGYTMNWVRQAPGKGLEWVGLINPYNGGTIYNQKFKGRFTLSVDKSKSTAYLQMNSLRAEDTAVYYCARDYGFVLDYWGRGTLVTVSSASTKGPSVFPLAPSSKSTSGGTAALGCLVKDYFPEPVTVSWNSGALTSGVHTFPAVLQSSGLYSLSSVVTVPSSSLGTQTYICNVNHKPSNTKVDKRVEPKSCDKTHTCPPCPAPELLGGPSVFLFPPKPKDTLMISRTPEVTCVVVDVSHEDPEVKFNWYVDGVEVHNAKTKPREEQYNSTYRVVSVLTVLHQDWLNGKEYKCKVSNKALPAPIEKTISKAKGQPREPQVYTLPPSREEMTKNQVSLTCLVKGFYPSDIAVEWESNGQPENNYKTTPPVLDSDGSFFLYSKLTVDKSRWQQGNVFSCSVMHEALHNHYTQKSLSLSPGK

SEQ ID NO: 3 - DNA, 642 bp, synthetic construct
  source 1..642: mol_type = other DNA
gacatccagctgacccagtctccatcctctctgtctgcctctgtgggcgacagagtgacaattacctgctccgcctcctcctccgtgtcctacctgcattggttccagcagaagcctggcaaggcccctaagctgctggtgtactccacctccaatctgccttccggcgtgccctctagattctccggatctggctctggcaccgactataccctgacaatctccagcctgcagcctgaggacttcgccacctactactgccagcagcggtctatctaccctccttggacctttggccagggcaccaagctggaaatcaagcgtacggtggccgctccttccgtgttcatcttcccaccttccgacgagcagctgaagtccggcacagcttctgtcgtgtgcctgctgaacaacttctaccctcgggaagccaaggtgcagtggaaggtggacaatgccctgcagtccggcaactcccaagagtctgtgaccgagcaggactccaaggacagcacctacagcctgtcctccacactgaccctgtccaaggccgactacgagaagcacaaggtgtacgcctgcgaagtgacccatcagggcctgtctagccctgtgaccaagtctttcaaccggggcgagtgc

SEQ ID NO: 4 - protein, 214 aa, synthetic construct
DIQLTQSPSSLSASVGDRVTITCSASSSVSYLHWFQQKPGKAPKLLVYSTSNLPSGVPSRFSGSGSGTDYTLTISSLQPEDFATYYCQQRSIYPPWTFGQGTKLEIKRTVAAPSVFIFPPSDEQLKSGTASVVCLLNNFYPREAKVQWKVDNALQSGNSQESVTEQDSKDSTYSLSSTLTLSKADYEKHKVYACEVTHQGLSSPVTKSFNRGEC

SEQ ID NO: 5 - DNA, 1341 bp, synthetic construct
  source 1..1341: mol_type = other DNA
caggtgcagctggtggaatctggtggcggagttgttcagcctggcggctctctgagactgtcctgcaaggcttccggctactccttcaccggctacaccatgaactgggtccgacaggctcctggcaaaggcctggaatgggtcggactgatcaacccctataacggcggcaccatctacaaccagaagttcaagggcagattcaccctgtccgtggacaagtccaagtccaccgcctacctgcagatgaactccctgagagccgaggacaccgccgtgtactactgcgctagagactacggctacgtgctggactattggggcagaggcacactggtcaccgtgtcctctgctagcacaaagggacctagcgtatttccattggctcctagcagcaaatccacaagtggtggaactgctgcactgggttgtctggttaaggattatttcccagagccagtcacagtttcctggaactctggggcactgacctccggagtgcacacattcccagccgtacttcaatccagtggtctctacagcctttcttcagtagtaaccgttccatcttctagcctcggaacccaaacttatatttgcaatgtgaatcacaagccttctaacactaaggttgataaacgagtcgaaccaaaatcctgcgataagacccacacttgcccaccttgccccgcaccagaattgttgggtggaccctctgtgttcctctttccacctaaacctaaggacactcttatgatctcacgcactcctgaagtaacctgtgtagtagtagacgtaagccatgaagaccccgaagtgaagttcaactggtatgttgatggtgtcgaagtgcataatgccaagactaaaccccgagaagaacagtataattctacttatagagtggtgtcagtgttgacagttctgcaccaagattggctcaatggtaaggagtacaaatgcaaggtgtcaaacaaggcactgccagcccctattgaaaagaccatcagcaaggccaagggccaacctcgagagccacaagtctacactctccctccttcacgtgaggagatgactaagaatcaggtttctctgacatgtttggtaaagggtttctacccaagcgacatagctgtggagtgggaatctaatggtcaaccagagaacaattacaaaaccaccccacccgttctcgactctgacggcagtttcttcctgtatagcaaacttactgtggataaatcccgatggcaacaaggcaacgtcttttcttgttccgtgatgcatgaggcacttcataaccactatacacaaaagagtttgtctttgtctccaggaaaa

SEQ ID NO: 6 - protein, 447 aa, synthetic construct
QVQLVESGGGVVQPGGSLRLSCKASGYSFTGYTMNWVRQAPGKGLEWVGLINPYNGGTIYNQKFKGRFTLSVDKSKSTAYLQMNSLRAEDTAVYYCARDYGYVLDYWGRGTLVTVSSASTKGPSVFPLAPSSKSTSGGTAALGCLVKDYFPEPVTVSWNSGALTSGVHTFPAVLQSSGLYSLSSVVTVPSSSLGTQTYICNVNHKPSNTKVDKRVEPKSCDKTHTCPPCPAPELLGGPSVFLFPPKPKDTLMISRTPEVTCVVVDVSHEDPEVKFNWYVDGVEVHNAKTKPREEQYNSTYRVVSVLTVLHQDWLNGKEYKCKVSNKALPAPIEKTISKAKGQPREPQVYTLPPSREEMTKNQVSLTCLVKGFYPSDIAVEWESNGQPENNYKTTPPVLDSDGSFFLYSKLTVDKSRWQQGNVFSCSVMHEALHNHYTQKSLSLSPGK

SEQ ID NO: 7 - DNA, 642 bp, synthetic construct; identical to SEQ ID NO: 3
  source 1..642: mol_type = other DNA

SEQ ID NO: 8 - protein, 214 aa, synthetic construct; identical to SEQ ID NO: 4